European Patent Application EP 4 685 233 A1, published January 28, 2026. Title: PROTEASE-VARIANTEN MIT VERBESSERTER LAGERSTABILITÄT. Applicant: Henkel AG & Co. KGaA. Application EP. The sequence listing filed with the application follows.

SEQUENCE LISTING (1 sequence)

SEQ ID NO: 1 - protein, 269 aa, Halalkalibacter okhensis
NQTIPWGITRVQAPAAINRGFTGAGVRVAVLDTGISNHPDLNIRGGVSFVPGESTYQDGNGHGTHVAGTIAALNNSIGVVGVAPNTELYAVKVLGANGSGSISSIAQGLQWTAQNNIHVANLSLGSPTGSQTLELAVNQATSAGVLVVAASGNNGSGTISYPARYANALAVGATDQNNNRASFSQYGTGLNIVAPGVGVQSTYPGNRYASLSGTSMATPHVAGVAALVKQKNPGWSNTQIRQHLLNTATPLGSSNQYGSGLVNAEAATR